European Patent Application EP 4 474 483 A1, published December 11, 2024. Title: METHOD FOR SCREENING SUBSTANCE SUPPRESSING 4-METHYLACETOPHENONE FLAVOR AND METHOD FOR SUPPRESSING 4-METHYLACETOPHENONE FLAVOR. Applicant: 味の素株式会社. The sequence listing filed with the application follows.

SEQUENCE LISTING (2 sequences)

SEQ ID NO: 1 - DNA, 1017 bp, Homo sapiens
  source 1..1017: mol_type = genomic DNA
atggggactggaaatgacaccactgtggtagagtttactcttttggggttatctgaggatactacagtttgtgctattttatttcttgtgtttctaggaatttatgttgtcaccttaatgggtaatatcagcataattgtattgatcagaagaagtcatcatcttcatacacccatgtacattttcctctgccatttggcctttgtagacattgggtactcctcatcagtcacacctgtcatgctcatgagcttcctaaggaaagaaacctctctccctgttgctggttgtgtggcccagctctgttctgtagtgacgtttggtacggccgagtgcttcctgctggctgccatggcctatgatcgctatgtggccatctgctcacccctgctctactctacctgcatgtcccctggagtctgcatcatcttagtgggcatgtcctacctgggtggatgtgtgaatgcttggacattcattggctgcttattaagactgtccttctgtgggccaaataaagtcaatcactttttctgtgactattcaccacttttgaagcttgcttgttcccatgattttacttttgaaataattccagctatctcttctggatctatcattgtggccactgtgtgtgtcatagccatatcctacatctatatcctcatcaccatcctgaagatgcactccaccaagggccgccacaaggccttctccacctgcacctcccacctcactgcagtcactctgttctatgggaccattaccttcatttatgtgatgcccaagtccagctactcaactgaccagaacaaggtggtgtctgtgttctacaccgtggtgattcccatgttgaaccccctgatctacagcctcaggaacaaggagattaagggggctctgaagagagagcttagaataaaaatattttctgtttaaacgaattcgagctcggtacccggggatcctctagagtcgacctgcaggcatgcaagctgatccggctgctaacaaagc

SEQ ID NO: 2 - protein, 312 aa, Homo sapiens
MGTGNDTTVVEFTLLGLSEDTTVCAILFLVFLGIYVVTLMGNISIIVLIRRSHHLHTPMYIFLCHLAFVDIGYSSSVTPVMLMSFLRKETSLPVAGCVAQLCSVVTFGTAECFLLAAMAYDRYVAICSPLLYSTCMSPGVCIILVGMSYLGGCVNAWTFIGCLLRLSFCGPNKVNHFFCDYSPLLKLACSHDFTFEIIPAISSGSIIVATVCVIAISYIYILITILKMHSTKGRHKAFSTCTSHLTAVTLFYGTITFIYVMPKSSYSTDQNKVVSVFYTVVIPMLNPLIYSLRNKEIKGALKRELRIKIFSV